European Patent Specification EP 4 108 783 B1, published February 21, 2024. Title: SPATIAL SEQUENCING WITH MICTAG. Applicant: Miltenyi Biotec B.V. & Co. KG. The sequence listing filed with the application follows.

SEQUENCE LISTING (4 sequences)

SEQ ID NO: 1 - RNA, 15 nt, Homo sapiens
gctagtactcgagcc

SEQ ID NO: 2 - RNA, 16 nt, Homo sapiens
gcaacggcctagcctg

SEQ ID NO: 3 - RNA, 10 nt, Homo sapiens
cgcaaaggct

SEQ ID NO: 4 - RNA, 41 nt, Homo sapiens
tgatcatgagctcggcgttgccggatcggtcgcgtttccga